European Patent Specification EP 3 867 366 B1, published April 30, 2025. Title: CRISPR system for genome editing. Applicant: UNIVERSITA’ DEGLI STUDI DI SIENA; ISTITUTO PER LO STUDIO, LA PREVENZIONE E LA RETE ONCOLOGICA (ISPRO); UNIVERSITA’ DEGLI STUDI DI FIRENZE. The sequence listing filed with the application follows.

SEQUENCE LISTING (8 sequences)

SEQ ID NO: 1 - DNA, 13710 bp, Artificial sequence
  CRISPR-Cas viral vector
caaaagaatagaccgagatagggttgagtgttgttccagtttggaacaagagtccactattaaagaacgtggactccaacgtcaaagggcgaaaaaccgtctatcagggcgatggcccactacgtgaaccatcaccctaatcaagttttttggggtcgaggtgccgtaaagcactaaatcggaaccctaaagggagcccccgatttagagcttgacggggaaagccggcgaacgtggcgagaaaggaagggaagaaagcgaaaggagcgggcgctagggcgctggcaagtgtagcggtcacgctgcgcgtaaccaccacacccgccgcgcttaatgcgccgctacagggcgcgtggggataccccctagagccccagctggttctttccgcctcagaagccatagagcccaccgcatccccagcatgcctgctattgtcttcccaatcctcccccttgctgtcctgccccaccccaccccccagaatagaatgacacctactcagacaatgcgatgcaatttcctcattttattaggaaaggacagtgggagtggcaccttccagggtcaaggaaggcacgggggaggggcaaacaacagatggctggcaactagaaggcacagtcgaggctgatcagcgggtttaaacgggccctgctagagattttccacactgactaaaagggtctgagggatctctagttaccagagtcacacaacagacgggcacacactacttgaagcactcaaggcaagctttattgaggcttaagcagtgggttccctagttagccagagagctcccaggctcagatctggtctaaccagagagacccagtacaagcaaaaagcagatcttgtcttcgttgggagtgaattagcccttccagtccccccttttcttttaaaaagtggctaagatctacagctgccttgtaagtcattggtcttaaagtcgacgcggggaggcggcccaaagggagatccgactcgtctgagggcgaaggcgaagacgcggaagaggccgcagagccggcagcaggccctagagagggcctatttcccatgattccttcatatttgcatatacgatacaaggctgttagagagataattggaattaatttgactgtaaacacaaagatattagtacaaaatacgtgacgtagaaagtaataatttcttgggtagtttgcagttttaaaattatgttttaaaatggactatcatatgcttaccgtaacttgaaagtatttcgatttcttggctttatatatcttgtggaaaggacgaaacaccgtaatttctactcttgtagattctgctaatcctgttaccagccctaatttctactcttgtagattcagcagcgctcatggtgggggcttttttctattgcatgaagaatctgcttagggttaggcgttttgcgctgcttcgcgatgtacgggccagatatacgcgggtaccctctagaactagtggatcatttgtcgacgaattctatctctgctaatcctgttaccagcccggatccatggaaagaagaagcgcaaggtgggaagcggagctactaacttcagcctgctgaagcaggctggcgacgtggaggagaaccctggacctatggtgagcaagggcgaggagctgttcaccggggtggtgcccatcctggtcgagctggacggcgacgtaaacggccacaagttcagcgtgtccggcgagggcgagggcgatgccacctacggcaagctgaccctgaagttcatctgcaccaccggcaagctgcccgtgccctggcccaccctcgtgaccaccctgacctacggcgtgcagtgcttcagccgctaccccgaccacatgaagcagcacgacttcttcaagtccgccatgcccgaaggctacgtccaggagcgcaccatcttcttcaaggacgacggcaactacaagacccgcgccgaggtgaagttcgagggcgacaccctggtgaaccgcatcgagctgaagggcatcgacttcaaggaggacggcaacatcctggggcacaagctggagtacaactacaacagccacaacgtctatatcatggccgacaagcagaagaacggcatcaaggtgaacttcaagatccgccacaacatcgaggacggcagcgtgcagctcgccgaccactaccagcagaacacccccatcggcgacggccccgtgctgctgcccgacaaccactacctgagcacccagtccgccctgagcaaagaccccaacgagaagcgcgatcacatggtcctgctggagttcgtgaccgccgccgggatcactctcggcatggacgagctgtacaagtactcagatctcgagctcaagcttgagggcagaggaagccttctaacatgcggggacgtggaggaaaatcccggccccatggcttcgtacccctgccatcaacacgcgtctgcgttcgaccaggctgcgcgttctcgcggccataacaaccgacgtacggcgttgcgccctcgccggcagcaaaaagccacggaagtccgcctggagcagaaaatgcccacgctactgcgggtttatatagacggtccccacgggatggggaaaaccaccaccacgcaactgctggtggccctgggttcgcgcgacgatatcgtctacgtacccgagccgatgacttactggcgggtgttgggggcttccgagacaatcgcgaacatctacaccacacaacaccgcctcgaccagggtgagatatcggccggggacgcggcggtggtaatgacaagcgcccagataacaatgggcatgccttatgccgtgaccgacgccgttctggctcctcatatcgggggggaggctgggagctcacatgccccgcccccggccctcaccctcatcttcgataggcatcccatcgccgccctcctgtgctacccggccgcgcgataccttatgggcagcatgaccccccaggccgtgctggcgttcgtggccctcatcccgccgaccttgcccggcacaaacatcgtgttgggggcccttccggaggacagacacatcgaccgcctggccaaacgccagcgccccggcgagcggcttgacctggctatgctggccgcgattcgccgcgtttatgggctgcttgccaatacggtgcggtatctgcagggcggcgggtcgtggcgggaggattggggacagctttcgggggcggccgtgccgccccagggtgccgagccccagagcaacgcgggcccacgaccccatatcggggacacgttatttaccctgtttcgggcccccgagttgctggcccccaacggcgacctgtataacgtgtttgcctgggctttggacgtcttggccaaacgcctccgtcccatgcacgtctttatcctggattacgaccaatcgcccgccggctgccgggacgccctgctgcaacttacctccgggatggtccagacccacgtcaccaccccaggctccataccgacgatctgcgacctggcgcgcacgtttgcccgggagatgggggaggctaactaaagcgtctctgtcgtgcccccaccatgagcgctgctgagatatctgcgagacggtcgactttagatccaagcttatcgataccggtacccgttacataacttacggtaaatggcccgcctggctgaccgcccaacgacccccgcccattgacgtcaatagtaacgccaatagggactttccattgacgtcaatgggtggagtatttacggtaaactgcccacttggcagtacatcaagtgtatcatatgccaagtacgccccctattgacgtcaatgacggtaaatggcccgcctggcattgtgcccagtacatgaccttatgggactttcctacttggcagtacatctacgtattagtcatcgctattaccatggtcgaggtgagccccacgttctgcttcactctccccatctcccccccctccccacccccaattttgtatttatttattttttaattattttgtgcagcgatgggggcggggggggggggggggcgcgcgccaggcggggcggggcggggcgaggggcggggcggggcgaggcggagaggtgcggcggcagccaatcagagcggcgcgctccgaaagtttccttttatggcgaggcggcggcggcggcggccctataaaaagcgaagcgcgcggcgggcgggagtcgctgcgcgctgccttcgccccgtgccccgctccgccgccgcctcgcgccgcccgccccggctctgactgaccgcgttactcccacaggtgagcgggcgggacggcccttctcctccgggctgtaattagctgagcaagaggtaagggtttaagggatggttggttggtggggtattaatgtttaattacctggagcacctgcctgaaatcactttttttcaggttggaccggctagcgtttaaacttaagcttgccaccatggccccaaagaagaagcggaaggtcggtatccacggagtcccagcagccacacagttcgagggctttaccaacctgtatcaggtgagcaagacactgcggtttgagctgatcccacagggcaagaccctgaagcacatccaggagcagggcttcatcgaggaggacaaggcccgcaatgatcactacaaggagctgaagcccatcatcgatcggatctacaagacctatgccgaccagtgcctgcagctggtgcagctggattgggagaacctgagcgccgccatcgactcctatagaaaggagaaaaccgaggagacaaggaacgccctgatcgaggagcaggccacatatcgcaatgccatccacgactacttcatcggccggacagacaacctgaccgatgccatcaataagagacacgccgagatctacaagggcctgttcaaggccgagctgtttaatggcaaggtgctgaagcagctgggcaccgtgaccacaaccgagcacgagaacgccctgctgcggagcttcgacaagtttacaacctacttctccggcttttatgagaacaggaagaacgtgttcagcgccgaggatatcagcacagccatcccacaccgcatcgtgcaggacaacttccccaagtttaaggagaattgtcacatcttcacacgcctgatcaccgccgtgcccagcctgcgggagcactttgagaacgtgaagaaggccatcggcatcttcgtgagcacctccatcgaggaggtgttttccttccctttttataaccagctgctgacacagacccagatcgacctgtataaccagctgctgggaggaatctctcgggaggcaggcaccgagaagatcaagggcctgaacgaggtgctgaatctggccatccagaagaatgatgagacagcccacatcatcgcctccctgccacacagattcatccccctgtttaagcagatcctgtccgataggaacaccctgtctttcatcctggaggagtttaagagcgacgaggaagtgatccagtccttctgcaagtacaagacactgctgagaaacgagaacgtgctggagacagccgaggccctgtttaacgagctgaacagcatcgacctgacacacatcttcatcagccacaagaagctggagacaatcagcagcgccctgtgcgaccactgggatacactgaggaatgccctgtatgagcggagaatctccgagctgacaggcaagatcaccaagtctgccaaggagaaggtgcagcgcagcctgaagcacgaggatatcaacctgcaggagatcatctctgccgcaggcaaggagctgagcgaggccttcaagcagaaaaccagcgagatcctgtcccacgcacacgccgccctggatcagccactgcctacaaccctgaagaagcaggaggagaaggagatcctgaagtctcagctggacagcctgctgggcctgtaccacctgctggactggtttgccgtggatgagtccaacgaggtggaccccgagttctctgcccggctgaccggcatcaagctggagatggagccttctctgagcttctacaacaaggccagaaattatgccaccaagaagccctactccgtggagaagttcaagctgaactttcagatgcctacactggcccggggctgggacgtgaatgtggagaagaaccggggcgccatcctgtttgtgaagaacggcctgtactatctgggcatcatgccaaagcagaagggcaggtataaggccctcagcttcgagcccacagagaaaaccagcgagggctttgataagatgtactatgactactttccggatgccgccaagatgatcccaaagtgcagcacccagctgaaggcggtgaccgcccactttcagacccacacaacccccatcctgctgtccaacaatttcatcgagcctctggagatcacaaaggagatctacgacctgaacaatcctgagaaggagccaaagaagtttcagacagcgtacgccaagaaaaccggcgaccagaagggctacagagaggccctgtgcaagtggatcgacttcacaagggattttctgtccaagtataccaagacaacctctatcgatctgtctagcctgcggccatcctctcagtataaggacctgggcgagtactatgccgagctgaatcccctgctgtaccacatcagcttccagagaatcgccgagaaggagatcatggatgccgtggagacaggcaagctgtacctgttccagatctataacaaggactttgccaagggccaccacggcaagcctaatctgcacacactgtattggaccggtctgttttctccagagaacctggccaagacaagcatcaagctgaatggccaggccgagctgttctaccgccctaagtccaggatgaagaggatggcacaccggctgggagagaagatgctgaacaagaagctgaaggatcagaaaaccccaatccccgacaccctgtaccaggagctgtacgactatgtgaatcacagactgtcccacgacctgtctgatgaggccagggccctgctgcccaacgtgatcaccaaggaggtgtctcacgagatcatcaaggataggcgctttaccagcgacaagttctttttccacgtgcctatcacactgaactatcaggccgccaattccccatctaagttcaaccagagggtgaatgcctacctgaaggagcaccccgagacacctatcatcggcatcgatcggggcgagagaaacctgatctatatcacagtgatcgactccaccggcaagatcctggagcagcggagcctgaacaccatccagcagtttgattaccagaagaagctggacaacagggagaaggagagggtggcagcaaggcaggcctggtctgtggtgggcacaatcaaggatctgaagcagggctatctgagccaggtcatccacgagatcgtggacctgatgatccactaccaggccgtggtggtgctggagaacctgaatttcggctttaagagcaagaggaccggcatcgccgagaaggccgtgtaccagcagttcgagaagatgctgatcgataagctgaattgcctggtgctgaaggactatccagcagagaaagtgggaggcgtgctgaacccataccagctgacagaccagttcacctcctttgccaagatgggcacccagtctggcttcctgttttacgtgcctgccccatatacatctaagatcgatcccctgaccggcttcgtggaccccttcgtgtggaaaaccatcaagaatcacgagagccgcaagcacttcctggagggcttcgactttctgcactacgacgtgaaaaccggcgacttcatcctgcactttaagatgaacagaaatctgtccttccagaggggcctgcccggctttatgcctgcatgggatatcgtgttcgagaagaacgagacacagtttgacgccaagggcacccctttcatcgccggcaagagaatcgtgccagtgatcgagaatcacagattcaccggcagataccgggacctgtatcctgccaacgagctgatcgccctgctggaggagaagggcatcgtgttcagggatggctccaacatcctgccaaagctgctggagaatgacgattctcacgccatcgacaccatggtggccctgatccgcagcgtgctgcagatgcggaactccaatgccgccacaggcgaggactatatcaacagccccgtgcgcgatctgaatggcgtgtgcttcgactcccggtttcagaacccagagtggcccatggacgccgatgccaatggcgcctaccacatcgccctgaagggccagctgctgctgaatcacctgaaggagagcaaggatctgaagctgcagaacggcatctccaatcaggactggctggcctacatccaggagctgcgcaacaaaaggccggcggccacgaaaaaggccggccaggcaaaaaagaaaaagggatcctacccatacgatgttccagattacgcttatccctacgacgtgcctgattatgcatacccatatgatgtccccgactatgcctaagaattcctagagctcgctgatcagcctcgactgtgccttctagttgccagccatctgttgtttgcccctcccccgtgccttccttgaccctggaaggtgccactcccactgtcctttcctaataaaatgaggaaattgcatcgcattgtctgagtaggtgtcattctattctggggggtggggtggggcaggacagcaagggggaggattgggaagagaatagcaggcatgctggggagcggccggccgcttgctgtgcggtggtcttacttttgttttgctcttcctctatcttgtctaaagcttccttggtgtcttttatctctatcctttgatgcacacaatagagggttgctactgtattatataatgatctaagttcttctgatcctgtctgaagggatggttgtagctgtcccagtatttgtctacagccttctgatgtttctaacaggccaggattaactgcgaatcgttctagctccctgcttgcccatactatatgttttaatttatattttttctttccccctggccttaaccgaattttttcccatcgcgatctaattctcccccgcttaatactgacgctctcgcacccatctctctccttctagcctccgctagtcaaaatttttggcgtactcaccagtcgccgcccctcgcctcttgccgtgcgcgcttcagcaagccgagtcctgcgtcgagagagctcctctggtttccctttcgctttcaagtccctgttcgggcgccactgctagagattttccacactgactaaaagggtctgagggatctctagttaccagagtcacacaacagacgggcacacactacttgaagcactcaaggcaagctttattgaggcttaagcagtgggttccctagttagccagagagctcccaggctcagatctggtctaaccagagagacccagtacaggcaaaacgcgctgcttatatagacctcccaccgtacacgcctaccgcccatttgcgtcaatggggcggagttgttacgacattttggaaagtcccgttgattttggtgccaaaacaaactcccattgacgtcaatggggtggagacttggaaatccccgtgagtcaaaccgctatccacgcccattgatgtactgccaaaaccgcatcaccatggtaatagcgatgactaatacgtagatgtactgccaagtaggaaagtcccataaggtcatgtactgggcataatgccaggcgggccatttaccgtcattgacgtcaatagggggcgtacttggcatatgatacacttgatgtactgccaagtgggcagtttaccgtaaatactccacccattgacgtcaatggaaagtccctattggcgttactatgggaacatacgtcattattgacgtcaatgggcgggggtcgttgggcggtcagccaggcgggccatttaccgtaagttatgtaacgcggaactccatatatgggctatgaactaatgaccccgtaattgattactattaataactagtcaataatcaatgtcaacgcgtatatctggcccgtacatcgcgaagcagcgcaaaacgcctaaccctaagcagattcttcatgcaattgtcggtcaagccttgccttgttgtagcttaaattttgctcgcgcactactcagcgacctccaacacacaagcagggagcagatactggcttaactatgcggcatcagagcagattgtactgagagtgcaccataggggatcgggagatctcccgatccgtcgacgtcaggtggcacttttcggggaaatgtgcgcggaacccctatttgtttatttttctaaatacattcaaatatgtatccgctcatgagacaataaccctgataaatgcttcaataatattgaaaaaggaagagtatgagtattcaacatttccgtgtcgcccttattcccttttttgcggcattttgccttcctgtttttgctcacccagaaacgctggtgaaagtaaaagatgctgaagatcagttgggtgcacgagtgggttacatcgaactggatctcaacagcggtaagatccttgagagttttcgccccgaagaacgttttccaatgatgagcacttttaaagttctgctatgtggcgcggtattatcccgtattgacgccgggcaagagcaactcggtcgccgcatacactattctcagaatgacttggttgagtactcaccagtcacagaaaagcatcttacggatggcatgacagtaagagaattatgcagtgctgccataaccatgagtgataacactgcggccaacttacttctgacaacgatcggaggaccgaaggagctaaccgcttttttgcacaacatgggggatcatgtaactcgccttgatcgttgggaaccggagctgaatgaagccataccaaacgacgagcgtgacaccacgatgcctgtagcaatggcaacaacgttgcgcaaactattaactggcgaactacttactctagcttcccggcaacaattaatagactggatggaggcggataaagttgcaggaccacttctgcgctcggcccttccggctggctggtttattgctgataaatctggagccggtgagcgtgggtctcgcggtatcattgcagcactggggccagatggtaagccctcccgtatcgtagttatctacacgacggggagtcaggcaactatggatgaacgaaatagacagatcgctgagataggtgcctcactgattaagcattggtaactgtcagaccaagtttactcatatatactttagattgatttaaaacttcatttttaatttaaaaggatctaggtgaagatcctttttgataatctcatgaccaaaatcccttaacgtgagttttcgttccactgagcgtcagaccccgtagaaaagatcaaaggatcttcttgagatcctttttttctgcgcgtaatctgctgcttgcaaacaaaaaaaccaccgctaccagcggtggtttgtttgccggatcaagagctaccaactctttttccgaaggtaactggcttcagcagagcgcagataccaaatactgttcttctagtgtagccgtagttaggccaccacttcaagaactctgtagcaccgcctacatacctcgctctgctaatcctgttaccagtggctgctgccagtggcgataagtcgtgtcttaccgggttggactcaagacgatagttaccggataaggcgcagcggtcgggctgaacggggggttcgtgcacacagcccagcttggagcgaacgacctacaccgaactgagatacctacagcgtgagctatgagaaagcgccacgcttcccgaagggagaaaggcggacaggtatccggtaagcggcagggtcggaacaggagagcgcacgagggagcttccagggggaaacgcctggtatctttatagtcctgtcgggtttcgccacctctgacttgagcgtcgatttttgtgatgctcgtcaggggggcggagcctatggaaaaacgccagcaacgcggcctttttacggttcctggccttttgctggccttttgctcacatgttctttcctgcgttatcccctgattctgtggataaccgtattaccgcctttgagtgagctgataccgctcgccgcagccgaacgaccgagcgcagcgagtcagtgagcgaggaagcggaagagcgcccaatacgcaaaccgcctctccccgcgcgttggccgattcattaatgcagctggcacgacaggtttcccgactggaaagcgggcagtgagcgcaacgcaattaatgtgagttagctcactcattaggcaccccaggctttacactttatgcttccggctcgtatgttgtgtggaattgtgagcggataacaatttcacacaggaaacagctatgaccatgattacgccaagctctagctagaggtcgacggtatacagacatgataagatacattgatgagtttggacaaaccacaactagaatgcagtgaaaaaaatgctttatttgtgaaatttgtgatgctattgctttatttgtaaccattataagctgcaataaacaagttggggtgggcgaagaactccagcatgagatccccgcgctggaggatcatccagccggcgtcccggaaaacgattccgaagcccaacctttcatagaaggcggcggtggaatcgaaatctcgtagcacgtgtcagtcctgctcctcggccacgaagtgcacgcagttgccggccgggtcgcgcagggcgaactcccgcccccacggctgctcgccgatctcggtcatggccggcccggaggcgtcccggaagttcgtggacacgacctccgaccactcggcgtacagctcgtccaggccgcgcacccacacccaggccagggtgttgtccggcaccacctggtcctggaccgcgctgatgaacagggtcacgtcgtcccggaccacaccggcgaagtcgtcctccacgaagtcccgggagaacccgagccggtcggtccagaactcgaccgctccggcgacgtcgcgcgcggtgagcaccggaacggcactggtcaacttggccatggtttagttcctcaccttgtcgtattatactatgccgatatactatgccgatgattaattgtcaacacgtgctgatcagatccgaaaatggatatacaagctcccgggagctttttgcaaaagcctaggcctccaaaaaagcctcctcactacttctggaatagctcagaggcagaggcggcctcggcctctgcataaataaaaaaaattagtcagccatggggcggagaatgggcggaactgggcggagttaggggcgggatgggcggagttaggggcgggactatggttgctgactaattgagatgcatgctttgcatacttctgcctgctggggagcctggggactttccacacctggttgctgactaattgagatgcatgctttgcatacttctgcctgctggggagcctggggactttccacaccctaactgacacacattccacagaattaattcgcgttaaatttttgttaaatcagctcattttttaaccaataggccgaaatcggcaaaatcccttataaat

SEQ ID NO: 2 - DNA, 43 bp, Artificial sequence
  Sequence encoding the first gRNA
taatttctactcttgtagattcagcagcgctcatggtgggggc

SEQ ID NO: 3 - DNA, 43 bp, Artificial sequence
  Sequence encoding the second gRNA
taatttctactcttgtagattctgctaatcctgttaccagccc

SEQ ID NO: 4 - DNA, 2035 bp, Artificial sequence
  EGFP-HSV-TK cassette
ggatccatggaaagaagaagcgcaaggtgggaagcggagctactaacttcagcctgctgaagcaggctggcgacgtggaggagaaccctggacctatggtgagcaagggcgaggagctgttcaccggggtggtgcccatcctggtcgagctggacggcgacgtaaacggccacaagttcagcgtgtccggcgagggcgagggcgatgccacctacggcaagctgaccctgaagttcatctgcaccaccggcaagctgcccgtgccctggcccaccctcgtgaccaccctgacctacggcgtgcagtgcttcagccgctaccccgaccacatgaagcagcacgacttcttcaagtccgccatgcccgaaggctacgtccaggagcgcaccatcttcttcaaggacgacggcaactacaagacccgcgccgaggtgaagttcgagggcgacaccctggtgaaccgcatcgagctgaagggcatcgacttcaaggaggacggcaacatcctggggcacaagctggagtacaactacaacagccacaacgtctatatcatggccgacaagcagaagaacggcatcaaggtgaacttcaagatccgccacaacatcgaggacggcagcgtgcagctcgccgaccactaccagcagaacacccccatcggcgacggccccgtgctgctgcccgacaaccactacctgagcacccagtccgccctgagcaaagaccccaacgagaagcgcgatcacatggtcctgctggagttcgtgaccgccgccgggatcactctcggcatggacgagctgtacaagtactcagatctcgagctcaagcttgagggcagaggaagccttctaacatgcggggacgtggaggaaaatcccggccccatggcttcgtacccctgccatcaacacgcgtctgcgttcgaccaggctgcgcgttctcgcggccataacaaccgacgtacggcgttgcgccctcgccggcagcaaaaagccacggaagtccgcctggagcagaaaatgcccacgctactgcgggtttatatagacggtccccacgggatggggaaaaccaccaccacgcaactgctggtggccctgggttcgcgcgacgatatcgtctacgtacccgagccgatgacttactggcgggtgttgggggcttccgagacaatcgcgaacatctacaccacacaacaccgcctcgaccagggtgagatatcggccggggacgcggcggtggtaatgacaagcgcccagataacaatgggcatgccttatgccgtgaccgacgccgttctggctcctcatatcgggggggaggctgggagctcacatgccccgcccccggccctcaccctcatcttcgataggcatcccatcgccgccctcctgtgctacccggccgcgcgataccttatgggcagcatgaccccccaggccgtgctggcgttcgtggccctcatcccgccgaccttgcccggcacaaacatcgtgttgggggcccttccggaggacagacacatcgaccgcctggccaaacgccagcgccccggcgagcggcttgacctggctatgctggccgcgattcgccgcgtttatgggctgcttgccaatacggtgcggtatctgcagggcggcgggtcgtggcgggaggattggggacagctttcgggggcggccgtgccgccccagggtgccgagccccagagcaacgcgggcccacgaccccatatcggggacacgttatttaccctgtttcgggcccccgagttgctggcccccaacggcgacctgtataacgtgtttgcctgggctttggacgtcttggccaaacgcctccgtcccatgcacgtctttatcctggattacgaccaatcgcccgccggctgccgggacgccctgctgcaacttacctccgggatggtccagacccacgtcaccaccccaggctccataccgacgatctgcgacctggcgcgcacgtttgcccgggagatgggggaggctaactaaagcgtctctgtcgt

SEQ ID NO: 5 - DNA, 4107 bp, Artificial sequence
  Sequence encoding Cas12a
atggccccaaagaagaagcggaaggtcggtatccacggagtcccagcagccacacagttcgagggctttaccaacctgtatcaggtgagcaagacactgcggtttgagctgatcccacagggcaagaccctgaagcacatccaggagcagggcttcatcgaggaggacaaggcccgcaatgatcactacaaggagctgaagcccatcatcgatcggatctacaagacctatgccgaccagtgcctgcagctggtgcagctggattgggagaacctgagcgccgccatcgactcctatagaaaggagaaaaccgaggagacaaggaacgccctgatcgaggagcaggccacatatcgcaatgccatccacgactacttcatcggccggacagacaacctgaccgatgccatcaataagagacacgccgagatctacaagggcctgttcaaggccgagctgtttaatggcaaggtgctgaagcagctgggcaccgtgaccacaaccgagcacgagaacgccctgctgcggagcttcgacaagtttacaacctacttctccggcttttatgagaacaggaagaacgtgttcagcgccgaggatatcagcacagccatcccacaccgcatcgtgcaggacaacttccccaagtttaaggagaattgtcacatcttcacacgcctgatcaccgccgtgcccagcctgcgggagcactttgagaacgtgaagaaggccatcggcatcttcgtgagcacctccatcgaggaggtgttttccttccctttttataaccagctgctgacacagacccagatcgacctgtataaccagctgctgggaggaatctctcgggaggcaggcaccgagaagatcaagggcctgaacgaggtgctgaatctggccatccagaagaatgatgagacagcccacatcatcgcctccctgccacacagattcatccccctgtttaagcagatcctgtccgataggaacaccctgtctttcatcctggaggagtttaagagcgacgaggaagtgatccagtccttctgcaagtacaagacactgctgagaaacgagaacgtgctggagacagccgaggccctgtttaacgagctgaacagcatcgacctgacacacatcttcatcagccacaagaagctggagacaatcagcagcgccctgtgcgaccactgggatacactgaggaatgccctgtatgagcggagaatctccgagctgacaggcaagatcaccaagtctgccaaggagaaggtgcagcgcagcctgaagcacgaggatatcaacctgcaggagatcatctctgccgcaggcaaggagctgagcgaggccttcaagcagaaaaccagcgagatcctgtcccacgcacacgccgccctggatcagccactgcctacaaccctgaagaagcaggaggagaaggagatcctgaagtctcagctggacagcctgctgggcctgtaccacctgctggactggtttgccgtggatgagtccaacgaggtggaccccgagttctctgcccggctgaccggcatcaagctggagatggagccttctctgagcttctacaacaaggccagaaattatgccaccaagaagccctactccgtggagaagttcaagctgaactttcagatgcctacactggcccggggctgggacgtgaatgtggagaagaaccggggcgccatcctgtttgtgaagaacggcctgtactatctgggcatcatgccaaagcagaagggcaggtataaggccctcagcttcgagcccacagagaaaaccagcgagggctttgataagatgtactatgactactttccggatgccgccaagatgatcccaaagtgcagcacccagctgaaggcggtgaccgcccactttcagacccacacaacccccatcctgctgtccaacaatttcatcgagcctctggagatcacaaaggagatctacgacctgaacaatcctgagaaggagccaaagaagtttcagacagcgtacgccaagaaaaccggcgaccagaagggctacagagaggccctgtgcaagtggatcgacttcacaagggattttctgtccaagtataccaagacaacctctatcgatctgtctagcctgcggccatcctctcagtataaggacctgggcgagtactatgccgagctgaatcccctgctgtaccacatcagcttccagagaatcgccgagaaggagatcatggatgccgtggagacaggcaagctgtacctgttccagatctataacaaggactttgccaagggccaccacggcaagcctaatctgcacacactgtattggaccggtctgttttctccagagaacctggccaagacaagcatcaagctgaatggccaggccgagctgttctaccgccctaagtccaggatgaagaggatggcacaccggctgggagagaagatgctgaacaagaagctgaaggatcagaaaaccccaatccccgacaccctgtaccaggagctgtacgactatgtgaatcacagactgtcccacgacctgtctgatgaggccagggccctgctgcccaacgtgatcaccaaggaggtgtctcacgagatcatcaaggataggcgctttaccagcgacaagttctttttccacgtgcctatcacactgaactatcaggccgccaattccccatctaagttcaaccagagggtgaatgcctacctgaaggagcaccccgagacacctatcatcggcatcgatcggggcgagagaaacctgatctatatcacagtgatcgactccaccggcaagatcctggagcagcggagcctgaacaccatccagcagtttgattaccagaagaagctggacaacagggagaaggagagggtggcagcaaggcaggcctggtctgtggtgggcacaatcaaggatctgaagcagggctatctgagccaggtcatccacgagatcgtggacctgatgatccactaccaggccgtggtggtgctggagaacctgaatttcggctttaagagcaagaggaccggcatcgccgagaaggccgtgtaccagcagttcgagaagatgctgatcgataagctgaattgcctggtgctgaaggactatccagcagagaaagtgggaggcgtgctgaacccataccagctgacagaccagttcacctcctttgccaagatgggcacccagtctggcttcctgttttacgtgcctgccccatatacatctaagatcgatcccctgaccggcttcgtggaccccttcgtgtggaaaaccatcaagaatcacgagagccgcaagcacttcctggagggcttcgactttctgcactacgacgtgaaaaccggcgacttcatcctgcactttaagatgaacagaaatctgtccttccagaggggcctgcccggctttatgcctgcatgggatatcgtgttcgagaagaacgagacacagtttgacgccaagggcacccctttcatcgccggcaagagaatcgtgccagtgatcgagaatcacagattcaccggcagataccgggacctgtatcctgccaacgagctgatcgccctgctggaggagaagggcatcgtgttcagggatggctccaacatcctgccaaagctgctggagaatgacgattctcacgccatcgacaccatggtggccctgatccgcagcgtgctgcagatgcggaactccaatgccgccacaggcgaggactatatcaacagccccgtgcgcgatctgaatggcgtgtgcttcgactcccggtttcagaacccagagtggcccatggacgccgatgccaatggcgcctaccacatcgccctgaagggccagctgctgctgaatcacctgaaggagagcaaggatctgaagctgcagaacggcatctccaatcaggactggctggcctacatccaggagctgcgcaacaaaaggccggcggccacgaaaaaggccggccaggcaaaaaagaaaaagggatcctacccatacgatgttccagattacgcttatccctacgacgtgcctgattatgcatacccatatgatgtccccgactatgcctaa

SEQ ID NO: 6 - DNA, 23 bp, Artificial sequence
  First target sequence
gcccccaccatgagcgctgctga

SEQ ID NO: 7 - DNA, 23 bp, Artificial sequence
  Second target sequence
tctgctaatcctgttaccagccc

SEQ ID NO: 8 - DNA, 249 bp, Artificial sequence
  U6 promoter
gagggcctatttcccatgattccttcatatttgcatatacgatacaaggctgttagagagataattggaattaatttgactgtaaacacaaagatattagtacaaaatacgtgacgtagaaagtaataatttcttgggtagtttgcagttttaaaattatgttttaaaatggactatcatatgcttaccgtaacttgaaagtatttcgatttcttggctttatatatcttgtggaaaggacgaaacacc